European Patent Application EP 4 806 992 A1, published September 16, 2026. Title: 암 치료용 신호물질 발현용 DNA 컨스트럭트, 및 이를 이용한 암 치료 방법. Applicant: 전남대학교 산학협력단. The sequence listing filed with the application follows.

SEQUENCE LISTING (48 sequences)

SEQ ID NO: 1 - DNA, 1083 bp, Escherichia coli
  source 1..1083: mol_type = other DNA
atggaaaaagagaaaaaaggggcgaaacacgagttagacctgtcatctatattgcagtttgttgctccgggtacaccgctcagagcggggatggaaaacgtcttgagagcaaatacaggcggtctgattgttgttggatataatgataaagtaaaagaagtggtggacggcggctttcacataaacacggctttttctccggcgcatttatatgagctggctaaaatggatggagcgatcattttaagtgattctggtcaaaagatcctatacgcgaatactcagctgatgccggatgccacaatttcttcatcagaaacaggaatgcggcacagaactgccgaaagagtagctaagcaaactggctgtcttgtaatcgccatttctgaaagaagaaatgtcataacgttatatcaggaaaacatgaagtatacactaaaagacataggatttattttaaccaaggcgaaccaagccattcaaacacttgaaaaatataagacaatcctcgataaaacgattaatgcactgaacgcgttagagtttgaggaacttgttaccttcagtgatgtcttgtctgtcatgcatcgttatgaaatggtactgagaatcaaaaacgaaattaatatgtatatcaaagagctggggacagaagggcatctgatcaaactgcaagtcattgaattgattacggatatggaagaagaggccgctttatttattaaggactatgtaaaagaaaagattaaagatccgtttgttctcttgaaggagctgcaggatatgtccagttatgatctgctggatgattccattgtgtataagcttctcggttaccctgcttctactaatcttgatgattatgtattgccgagaggatacaggctgttaaataagataccgcgtcttccgatgccgattgttgaaaatgttgtagaagcatttggagtcctgccaaggattattgaggcgagtgcagaagaattagatgaagtagagggaatcggtgaagtacgagcccaaaaaatcaaaaaaggattaaaacgcctgcaagagaagcattatttagacagacaactgtga

SEQ ID NO: 2 - DNA, 822 bp, Escherichia coli
  source 1..822: mol_type = other DNA
atggcttttgaggatatcccttttttgcagtacctcggcaatgccgttgatattctccttgtttggtatgtgatatataaattgattatggtgatacgcggcacgaaagcggttcagctgttaaaaggaattgtagtcatcgtgcttgttcgtatggccagccaatatttgggcctcagcacacttcaatggctgatggaccaagcgataacatggggatttttagcaattattattatttttcagcctgagctgagaagagcgcttgaacagctaggccgcggccgctttttttcgaggagcggcacgcctgttgaagaagcgcagcagaaaacgattgaggccattacaaaagcaatcaattatatggcgaaacgccgtataggcgccctgctgaccattgagcgggatactggaatgggcgattatattgagaccggcataccactaaatgccaaagtcagctctgagctgctgatcaatatttttattccaaacaccccgcttcatgacggtgcggtaattatgaaaaataatgaaattgccgcggccgcctgttatctgccgctttctgagagcccgtttatttcaaaagaactgggcacgcggcacagagcagctgtcggtatcagtgaagtaacagacagtttgacgattattgtgtctgaagagaccggcggcgtcagtgtggcaaagaacggcgaccttcacagagagcttacagaagaagcgctgaaagaaatgcttgaagccgagtttaagaaaaacaccagagacacttcttctaaccgctggtattggaggggcaggaaaaatggataa

SEQ ID NO: 3 - DNA, 624 bp, Escherichia coli
  source 1..624: mol_type = other DNA
atgaaggctatgcgctatgagcagatatcagaaaatgcgttcaaggggaaaatacaggtgtacttagagcaaatattaggtgatgcatctctaatcttgaaaacgcttcacgaaaaagaccagtgtctcctttgtgaattagatgatttggggcacgtttttcaggacatgcaggggattgcatcctccttttatttgcaatcatacattgaggaatttacgccggcatttattgagctggccaaggcgattaaagccttatcggaacataagcatggagctttaattgtgattgaaagagcagacccggttgaacgttttattcaaaaaggcacctccctacacgccgagatcagctcttcattaattgaaagcatcttttttcccggaaaccctcttcatgacggcgctttattagtgagggaaaacaaactcgtgtcagcagccaatgtgctcccgctgacgacgaaggaagtggatatccatttgggaacccggcaccgggcggctcttggtatgtcgggctatacggatgcactggtgctcgtggtttcagaggaaacagggaagatgtcgtttgccaaagacggtgtattatatccgttaatttcaccaagaacgtaa

SEQ ID NO: 4 - DNA, 1383 bp, Escherichia coli
  source 1..1383: mol_type = other DNA
atggagatgtattttaaaagaatgaaagatgagtggaccggacttgtcgaacaggcagatccgcccattcgtgctaaagccgcggaaattgccgttgcgcatgctcattatctgagtatcgagttttatcgaattgtccgcatcgacccgcatgccgaagaattcttgagtaatgaacaagttgagcggcagttgaagagtgcgatggaacgctggattattaacgtgctttctgcccaggttgacgatgtcgaaaggctaatacaaatccagcataccgtcgcggaagtgcatgcccgcataggaattccggtagaaattgtcgagatggggtttcgggtgctgaaaaaaatcctctatccggtgatcttctcttcggattattccgccgcagaaaaacttcaggtctaccatttctcgattaacagtattgatatcgcgatggaagtgatgactcgcgcgtttacctttagtgacagtagtgcctcaaaggaagatgaaaactatcgtatcttctcgttactggaaaacgccgaagaagaaaaagaacggcaaatagcctcaatactttcatgggaaatagatattatctataaaatcctgctggattctgatttaggcagtagtttgcctttaagccaggctgattttggcctgtggtttaaccataaaggtcgacattattttagtggtattgccgaagtaggccatatctcccgtctgattcaggatttcgacggtattttcaatcaaaccatgcgtaacaccagaaatttgaataacagaagtctgcgggtgaaatttttattacagataagaaataccgtatcgcaaattattaccttgctgcgtgaattgtttgaagaagtatcgcgccacgaagtcggtatggatgtactgacgaaattacttaaccgccgtttcctaccgactatcttcaaacgcgaaattgcccatgccaaccggaccggtacaccgctgtcagtgctgattattgacgttgataaattcaaagagatcaacgatacgtggggccataacactggtgatgaaattctgcgtaaagtctctcaggccttttatgacaacgtccgcagtagtgattatgttttccgctacgggggcgatgaatttatcattgttttgactgaagcttctgaaaacgaaacgttacgtaccgcagaacgtattcgcagtcgggtggagaaaaccaaactgaaagccgcaaacggcgaagatattgccctctcactttccatcggtgccgccatgtttaatggtcatcctgactatgagcgcctcattcaaatagccgatgaagctctgtatatcgccaaaagacgaggtagaaaccgtgttgaactctggaaagccagtctttag

SEQ ID NO: 5 - DNA, 1116 bp, Escherichia coli
  source 1..1116: mol_type = other DNA
atgttcccaaaaataatgaatgatgaaaactttttcaaaaaagcggcggcgcacggggaggaacctcctttaactcctcaaaacgaacatcagcggtccgggctgcgcttcgcccgtcgcgtcagactaccccgtgcggttggcctggctggcatgttcttaccgattgcttcaacgctggtttcacacccgccgccgggctggtggtggctggtgttggtcggctgggcgttcgtctggccgcatttagcctggcagatagcgagcagggccgtcgatccgcttagccgggaaatttacaacttaaaaaccgatgcagtattagcgggaatgtgggtaggcgtaatgggcgtaaacgtgctgccttccaccgcgatgttgatgattatgtgtctgaatttgatgggggcaggcggcccccgtctgtttgtcgcgggtctggtgttgatggtggtttcctgccttgtcaccctcgagctgacgggcattaccgtgtcgttcaatagtgcgccgctggaatggtggctctcccttcccattattgtcatttatcctctgctgtttggctgggtcagctaccagacggcaaccaaactggcggaacataaacgcaggttgcaggtcatgagtacccgcgacggcatgacgggcgtgtataaccgacgtcattgggaaactatgttacgcaatgaatttgataactgtcggcggcataatcgcgatgcaacgttactgattatcgatatcgaccatttcaagagcatcaacgatacctggggccatgatgtgggcgatgaagcgattgtggcgcttacccgacagttacaaattaccctgcgcggtagcgatgtgattggtcggtttggcggcgatgagtttgcagtaatcatgtccggtacgccagctgagagcgccattaccgccatgttacgggtgcatgaagggctaaatacattacgtttgccgaatacgccacaggtaactttacggattagtgtgggggttgcgccgctgaacccacaaatgagtcactatcgtgagtggttgaaatcggcagatttggcgctttacaaagcaaagaaagccggacgtaaccgcaccgaagtggcggcctga

SEQ ID NO: 6 - DNA, 891 bp, Escherichia coli
  source 1..891: mol_type = other DNA
atgatcaagaagacaacggaaattgatgccatcttgttaaatctcaataaggctatcgatgcccactaccagtggctggtgagtatgtttcacagcgtggtcgcgagagatgccagtaagccagaaataacggataaccattcttatggactgtgccagtttggtcggtggattgatcatctggggccactcgataacgatgaattaccttacgttcggctaatggattctgcccatcaacatatgcataactgtggtcgggaattaatgctggctattgttgaaaatcactggcaggacgcgcatttcgacgcctttcaggaggggttgctttcttttactgcggcattaaccgattacaaaatttatttgctgacgatccgtagcaatatggatgttttgacgggattgccgggtcgtcgggttcttgatgaatcctttgatcatcagttacgcaacgctgagcctctgaatctttatttaatgttgttggatattgaccgatttaaattggttaatgatacctacgggcatttaatcggcgatgtagtattacgcaccctggcaacttacttagccagttggacgcgtgattacgaaacggtttatcgctacgggggcgaagaatttatcattattgtcaaagcggctaatgatgaagaagcatgtcgtgcaggtgtcagaatttgccagttagtcgataaccatgccatcacacattctgaagggcatatcaacattaccgtgacagcaggtgtgagtcgcgcatttcctgaagagcctctggatgtggtcattggaagagcggaccgggcaatgtatgagggtaagcaaaccggaagaaatcgctgcatgtttattgacgaacaaaatgtgattaaccgagtttaa

SEQ ID NO: 7 - DNA, 1221 bp, Escherichia coli
  source 1..1221: mol_type = other DNA
atgaataaggaattttctctgtccaggccaacatttaaacgcacactacggcggattagtataatcagcgtgctgcttacaatgacattgatctggctattaatttgcgttgcgtctgtccttacgctcaaacagtatgcgcaaaagaatctcgatttgaccgccgccacaatggcccatagccttgaagcggcactggtattttccgataacgcggccgcagcggaaacgctcgccacactgggacgccagggacaattttcagcggcggaggtccgcgataaaaatggccgtactatcgcctcatggcgctatgatgcgcgagccgcagacgataagctcattggcttaattagccactggctttttccattgccggtatcacaacccgtctggcacaacggcagggccatcggcgaagtacggcttgtcgcccgcgacagccttattggtcattttatctggctatcgctggcagtgctgacaggatgtattctgctggcatccggcattgccctgctgctcacgcgttatttacacaatggcgttgtggatgcgctgcaaaatattactgaagttgtacacgacgttcgcactaaccgaaatttttcacgccgggtacctgatgagcgtattgcggaatttcacctgtttgcgcaggatttcaatagccttctggatgagatggaagaatggcagctacggcttcaggctaaaaatgcccagttactacgtaccgcgttgcacgatccgctgacggggcttgccaatcgcgcggcatttcgcagctgtattaacgcgctgatgaaggacaattccgctcgtagcagttcggcattgttatttctggatggcgataactttaaatatattaatgatacctggggacatgcggcaggcgaccgcgtacttatagaggttgccaaaagattagcggaattcggtggtagccgttatcagacttaccgactcggcggcgatgaatttgcgatggtgctttacgatgtacattcggaatatgaagtacaacgtatttgcgcagcgctatcccaggcgtttaatcgaccttttgaactgcataacggccagcgaataacgatgaccctgagtattggctttgcgctgacatgggaacatgccactgccgaaaaactacaagaactggccgatcgaaatatgtatcaggctaaacaccggcgtgcggagcgctcgctaaactaa

SEQ ID NO: 8 - DNA, 1113 bp, Escherichia coli
  source 1..1113: mol_type = other DNA
atgttcccaaaaataatgaatgatgaaaatttttaccgaaaagcggttgaacaggcggtagcgccgcctgaccctcctgatgatcgtcagcgctccgggttgcgcttcgcccggcgcatcaggctaccgcgtgcggtggggttaggggggatgtttttaccggtggccgccgtgttagtgacgcaacctgtctttggcggctggtggctattgctggtcggctggtcttttgtctggccgcatctggcatggcagtgggcggcgaaagcccttgatccgctacgccaggaaatttacaacctgaaagtggatgcgatcctctccggcatgtggatcgcgctgatgggcgtcaatatgttgcctgccgccgcgctgtttatgatgatgagcatgaatctgatgggcgctggcgggcggcggctattcactgtcggaatgggccttttgctggcgtcatgtctggtgacgttgcagcttgccgggctacccgtcgcgatgcgaagctcgtcgctggaagtcacgctctctttgcccgtcattatgttgtatccgcttctgttcgcctgggtaagttaccaaacggccattaaattagcggaacataagcgacgcttgcaggcgatgagctcgcgggatggcatgaccggcgtctataaccgacgccactgggaaattttattacgtaatgaattcgatcacagccgacgccaccatcgggaggcgacattgttgattatcgatatcgatcattttaagagcattaacgacacctggggacatgatgttggggatgaggctattatcgccctgacgcgtcaattacagataacgctacgcgggagtgatattatcgggcgctttggcggcgacgaatttgcggtgattatgtgcggaacgccggcagacagcgcgattaccgccatgtcgcgagtgcatgaacggctaaataccttacgcttgccgggcgcgccgcaggtcatgttacgtatcagcgtgggcgtggcgccgttaacgccacaaatcggtcattatcgggaatggctaaagtctgcggatatggcgctttacaaagcaaagaatgccggacgtaaccgcaccgaagtggcggcatga

SEQ ID NO: 9 - DNA, 1494 bp, Salmonella sp.
  source 1..1494: mol_type = other DNA
atgaatttgcatcataaagcgctcaggcactttatctcggcaagcgtcatcgttttgacatcgtccttcctgatttacgaacttattgccagcgacagggcaatgaatgcctatatgcgttatatcatggagagagccgattcgtcgtttttgtacgataagtaccagaatcagagcatcgccgcacatttgatgcgaacttttgaagcgccgggagaccccgtcaccgcagaaaaacaccgcgcgttttgcgacgcctttgaagctattaacggtacgcacggtgtcaacctgacccggcataattatccggcgctacatggtactctgcaaaccgccgctacacagtgtaccgataatcttgatgacgcccttttactgcctgcatttgatcaggcggtaagcatcaaccgttcgcaggacgaccatagtcacgggctgggcacactggagcttaaattccgttattacgttgatttaaataaacattatgtctatttctatgatttaatcaactcacggcgcttcgccatgcatcgttggacttttttacaaaaaggcacaatgggtattaacagaaaagatatagataaactttttaccggccgtacggttatttcaagtatctacatggatgatattactcaggaaaacgtcatgagttttttaacgccagtctatctggcgggatcgttaaaaggcatcgtgatggtggatgttaaccaggataatttaaaaaatattttttatacccaggaccgtccgctggtttggcgttatcttaacgtaacactaaaggatatggactccggaaaagaaattattattaatcaaagcaaaaataatctgtttcaatatgtgaattatagccatgatatccctggtgggctgcgcgtttcgttgtcccttgatttaacctatttccttgtctcgtcctggaaagcgctggccttttacttactggcaacggcgctcctgcttaatatggtacggatgcactttcggctttatcgcaacgtcacacgcgaaaatattagcgatgccatgaccgggctttacaaccgtaaaatattaacaccggtgctggaacagcgactgcaacgcctggtcaataccgggacgccggtgacatttgtcgctattgattgcgataggttaaaactgatcaacgatacccaggggcaccaggaaggcgaccgaattataaccctgttggcgaaagcgattaaaacatcgattcgtaaaagcgattacgccattcgcctcggcggcgatgagttctgtattattcttgttgattacgcggcggatttggctatccatctgccggagcgtattattcgtaacctgcaaattatcgcaccggataagacagtccatttttctgccgggatttataatatgcagcccaatgatacgattaatgatgcctaccaggcttccgatgcgcagctctatctgaacaaacaacaaaaacaacatcgttcatcatag

SEQ ID NO: 10 - DNA, 1569 bp, Escherichia coli
  source 1..1569: mol_type = other DNA
atgcagccttggcacggaaaggccatgcagagagcttccgaggccggagccactgcccccaaggcttccgcacggaatgccaggggcgccccgatggatcccaccgagtctccggctgcccccgaggccgccctgcctaaggcgggaaagttcggccccgccaggaagtcgggatcccggcagaaaaagagcgccccggacacccaggagaggccgcccgtccgcgcaactggggcccgcgccaaaaaggcccctcagcgcgcccaggacacgcagccgtctgacgccaccagcgcccctggggcagaggggctggagcctcctgcggctcgggagccggctctttccagggctggttcttgccgccagaggggcgcgcgctgctccacgaagccaagacctccgcccgggccctgggacgtgcccagccccggcctgccggtctcggcccccattctcgtacggagggatgcggcgcctggggcctcgaagctccgggcggttttggagaagttgaagctcagccgcgatgatatctccacggcggcggggatggtgaaaggggttgtggaccacctgctgctcagactgaagtgcgactccgcgttcagaggcgtcgggctgctgaacaccgggagctactatgagcacgtgaagatttctgcacctaatgaatttgatgtcatgtttaaactggaagtccccagaattcaactagaagaatattccaacactcgtgcatattactttgtgaaatttaaaagaaatccgaaagaaaatcctctgagtcagtttttagaaggtgaaatattatcagcttctaagatgctgtcaaagtttaggaaaatcattaaggaagaaattaacgacattaaagatacagatgtcatcatgaagaggaaaagaggagggagccctgctgtaacacttcttattagtgaaaaaatatctgtggatataaccctggctttggaatcaaaaagtagctggcctgctagcacccaagaaggcctgcgcattcaaaactggctttcagcaaaagttaggaagcaactacgactaaagccattttaccttgtacccaagcatgcaaaggaaggaaatggtttccaagaagaaacatggcggctatccttctctcacatcgaaaaggaaattttgaacaatcatggaaaatctaaaacgtgctgtgaaaacaaagaagagaaatgttgcaggaaagattgtttaaaactaatgaaataccttttagaacagctgaaagaaaggtttaaagacaaaaaacatctggataaattctcttcttatcatgtgaaaactgccttctttcacgtatgtacccagaaccctcaagacagtcagtgggaccgcaaagacctgggcctctgctttgataactgcgtgacatactttcttcagtgcctcaggacagaaaaacttgagaattattttattcctgaattcaatctattctctagcaacttaattgacaaaagaagtaaagaatttctgacaaagcaaattgaatatgaaagaaacaatgagtttccagtttttgatgaattttga

SEQ ID NO: 11 - DNA, 1071 bp, Escherichia coli
  source 1..1071: mol_type = other DNA
atggaagatccgcgtagaaggacgacggcgccacgcgctaagaagccgtccgcgaagcgcgccccgacgcagcccagcaggaccagggcccacgcggaaagctgcggcccgcaaaggggggctcgatcgcggcgggcggagcgtgacggggacaccacggagaagccacgtgccccagggccccgagtgcatccagcaagggccactgagctcaccaaagatgcacagccctcggccatggacgcggcaggagccaccgcgcggcctgccgtccgggtgccccagcagcaggccatcctggatccggagctgcccgccgtacgggagccccagccgcccgcggatcccgaggcgcggaaagtcgtaaggggacctagccacagaaggggcgcgcgctccaccgggcagcccagagcgccgcgagggtccaggaaggaaccggacaagctaaagaaggtgctggacaaattgagattgaaacgcaaagatatctcggaggcggccgagacggtgaataaagttgtggaacgcctgctgcgcagaatgcagaaacgggagtcggagttcaaaggtgtggagcagctgaacactggcagctactatgaacatgtgaagatttctgctcctaatgaatttgatgttatgtttaaactggaagtccccaggattgagctacaagaatattatgaaacaggtgctttctatcttgtgaaattcaaaagaattccacgaggaaatccgctgagtcatttcttagaaggggaagtattatcagctaccaagatgctgtcaaagtttaggaaaatcattaaagaagaagttaaagaaatcaaagatatagatgtcagtgtggagaaggaaaaaccaggaagccctgctgtaacacttcttatcaggaaccctgaagaaatctctgtggatataattctggctttggagtcaaaaggcagctggcctattagtaccaaagaaggactacctattcaaggctggctgggcacaaaagtgaggaccaatctaagagcgagagccgttttatctcgtacccaagaatgcaaaggatggaaatag

SEQ ID NO: 12 - DNA, 36 bp, synthetic construct
  source 1..36: mol_type = other DNA
aaaggcctaaagaggagaaagctagcatggaaaaag

SEQ ID NO: 13 - DNA, 58 bp, synthetic construct
  source 1..58: mol_type = other DNA
ggactagtttagtgatggtgatggtgatgcagttgtctgtctaaataatgcttctctt

SEQ ID NO: 14 - DNA, 34 bp, synthetic construct
  source 1..34: mol_type = other DNA
aaaggcctaaagaggagaaagctagcatggcttt

SEQ ID NO: 15 - DNA, 37 bp, synthetic construct
  source 1..37: mol_type = other DNA
ggactagtttagtgatggtgatggtgatgtccatttt

SEQ ID NO: 16 - DNA, 55 bp, synthetic construct
  source 1..55: mol_type = other DNA
aaaggcctaaagaggagaaagctagcatgaaggctatgcgctatgagcagatatc

SEQ ID NO: 17 - DNA, 46 bp, synthetic construct
  source 1..46: mol_type = other DNA
ggccgacgtcgacttacgttcttggtgaaattaacggatataatac

SEQ ID NO: 18 - DNA, 61 bp, synthetic construct
  source 1..61: mol_type = other DNA
aaactagtaaagaggagaaagctagcatggagatgtattttaaaagaatgaaagatgagtg

SEQ ID NO: 19 - DNA, 54 bp, synthetic construct
  source 1..54: mol_type = other DNA
gggagctcttagtgatggtgatggtgatgaagactggctttccagagttcaaca

SEQ ID NO: 20 - DNA, 66 bp, synthetic construct
  source 1..66: mol_type = other DNA
aaaggcctaaagaggagaaagctagcatgttcccaaaaataatgaatgatgaaaactttttcaaaa

SEQ ID NO: 21 - DNA, 46 bp, synthetic construct
  source 1..46: mol_type = other DNA
ggactagtttagtgatggtgatggtgatgggccgccacttcggtgc

SEQ ID NO: 22 - DNA, 55 bp, synthetic construct
  source 1..55: mol_type = other DNA
aaaggcctaaagaggagaaagctagcatgatcaagaagacaacggaaattgatgc

SEQ ID NO: 23 - DNA, 61 bp, synthetic construct
  source 1..61: mol_type = other DNA
ggactagtttagtgatggtgatggtgatgaactcggttaatcacattttgttcgtcaataa

SEQ ID NO: 24 - DNA, 54 bp, synthetic construct
  source 1..54: mol_type = other DNA
aaaggcctaaagaggagaaagctagcatgaataaggaattttctctgtccaggc

SEQ ID NO: 25 - DNA, 48 bp, synthetic construct
  source 1..48: mol_type = other DNA
ggactagtttagtgatggtgatggtgatggtttagcgagcgctccgca

SEQ ID NO: 26 - DNA, 63 bp, synthetic construct
  source 1..63: mol_type = other DNA
aaaggcctaaagaggagaaagctagcatgttcccaaaaataatgaatgatgaaaatttttacc

SEQ ID NO: 27 - DNA, 47 bp, synthetic construct
  source 1..47: mol_type = other DNA
ggactagtttagtgatggtgatggtgatgtgccgccacttcggtgcg

SEQ ID NO: 28 - DNA, 53 bp, synthetic construct
  source 1..53: mol_type = other DNA
aaaggcctaaagaggagaaagctagcatgaatttgcatcataaagcgctcagg

SEQ ID NO: 29 - DNA, 61 bp, synthetic construct
  source 1..61: mol_type = other DNA
ggactagtttagtgatggtgatggtgatgtgatgaacgatgttgtttttgttgtttgttca

SEQ ID NO: 30 - DNA, 47 bp, synthetic construct
  source 1..47: mol_type = other DNA
aaactagtaaagaggagaaagctagcatgcagccttggcacggaaag

SEQ ID NO: 31 - DNA, 60 bp, synthetic construct
  source 1..60: mol_type = other DNA
gggagctcttagtgatggtgatggtgatgaaattcatcaaaaactggaaactcattgttt

SEQ ID NO: 32 - DNA, 51 bp, synthetic construct
  source 1..51: mol_type = other DNA
aaaggcctaaagaggagaaagctagcatggaagatccgcgtagaaggacga

SEQ ID NO: 33 - DNA, 56 bp, synthetic construct
  source 1..56: mol_type = other DNA
gggagctcttagtgatggtgatggtgatgtttccatcctttgcattcttgggtacg

SEQ ID NO: 34 - DNA, 66 bp, synthetic construct
  source 1..66: mol_type = other DNA
atgaagaagaccgttctcgctttgtctttgctgataggtctgggcgcgacggcggccagttacgcc

SEQ ID NO: 35 - DNA, 60 bp, synthetic construct
  source 1..60: mol_type = other DNA
atgattcgtcatatcgccatttttctttgttctttattgatgtgcagcaccacttttgcc

SEQ ID NO: 36 - DNA, 63 bp, synthetic construct
  source 1..63: mol_type = other DNA
atgcaaaaatacgcgcttcacgcttacccagttatggccctgatggtcgcgacgctgacagga

SEQ ID NO: 37 - DNA, 60 bp, synthetic construct
  source 1..60: mol_type = other DNA
atggtgtttaaagctcttgcaggaatcgttctggcactggttgccactctggcgcacgcc

SEQ ID NO: 38 - DNA, 66 bp, synthetic construct
  source 1..66: mol_type = other DNA
atgaaacgacatatactggctaccgtgatagcatctcttgttgcagccccggcaatggcgctggcc

SEQ ID NO: 39 - DNA, 63 bp, synthetic construct
  source 1..63: mol_type = other DNA
atgaaccgtactaaccagctgatcttaggtgcagtagttctgggttccacgttactggcaggt

SEQ ID NO: 40 - DNA, 90 bp, synthetic construct
  source 1..90: mol_type = other DNA
atgttgaaaaaattaaagattaattatctgttcatcggcatattgacgctgctgctggcagcagccctttggccctcaatcccctggttc

SEQ ID NO: 41 - DNA, 63 bp, synthetic construct
  source 1..63: mol_type = other DNA
atgaaaaagacagctatcgcgattgcagtggcactggctggtttcgctaccgtagcgcaggcc

SEQ ID NO: 42 - DNA, 63 bp, synthetic construct
  source 1..63: mol_type = other DNA
atgaaacttaagttagtggcagtggcagtgacttccctgttggcagcaggcgttgtaaatgca

SEQ ID NO: 43 - DNA, 66 bp, synthetic construct
  source 1..66: mol_type = other DNA
atgatgaagcgcaaaatcctggcagcggtgatccctgccctgctggctgctgcaaccgcaaacgca

SEQ ID NO: 44 - DNA, 66 bp, synthetic construct
  source 1..66: mol_type = other DNA
atgaaatacctgctgccgaccgctgctgctggtctgctgctcctcgctgcccagccggcgatggcc

SEQ ID NO: 45 - DNA, 66 bp, synthetic construct
  source 1..66: mol_type = other DNA
atgtacagaaaaagcacacttgcgatgcttatcgctttgctaaccagcgctgcctcagcccatgcg

SEQ ID NO: 46 - DNA, 60 bp, synthetic construct
  source 1..60: mol_type = other DNA
atgaaatacacaatattgtcgctggtagctggtgcgctcatcagttgttcagcaatggca

SEQ ID NO: 47 - DNA, 66 bp, synthetic construct
  source 1..66: mol_type = other DNA
atgaaaaaaactttactcgcagtcagcgcagcgctggcgctcacctcatcttttactgctaacgca

SEQ ID NO: 48 - DNA, 75 bp, synthetic construct
  source 1..75: mol_type = other DNA
atgaaatttttgaaacggggtgtggcgctggcgttactggcggcgttcgcgctgacgactcagcctgcacaggct